European Patent Application EP 4 279 585 A1, published November 22, 2023. Title: CD7-TARGETED ENGINEERED IMMUNE CELL, CHIMERIC ANTIGEN RECEPTOR, CD7 BLOCKING MOLECULE AND USE THEREOF. Applicant: SHANGHAI YAKE BIOTECHNOLOGY LTD. The sequence listing filed with the application follows.

SEQUENCE LISTING (18 sequences)

SEQ ID NO: 1 - protein, 69 aa, Artificial sequence
TTTPAPAPPTPAPTIASGPLSLAPGACAPAAGGAVHTAGLAPACAITITAPLAGTCGVLLLSLVITLTC

SEQ ID NO: 2 - protein, 42 aa, Artificial sequence
LAGALLLLTIPLGPPMAPVGTTGGGAGCSCAPPGGGGGGCGL

SEQ ID NO: 3 - protein, 107 aa, Artificial sequence
IGVMTPPPTLAAGLSAGTIIHVLGLHLCPSPLPPGPSLPPTVLVVVGGVLACTSLLVTVAPIIPTVASLASALLHSATMAMTPAAPGPTALHTGPTAPPAAPAATAS

SEQ ID NO: 4 - protein, 112 aa, Artificial sequence
AVLPSASAAAPATGGGGAGLTAGLALGAAGGTAVLALAAGAAPGMGGLPAALAPGGGLTAGLGLALMAGATSGIGMLGGAAAGLGHAGLTGGLSTATLATTAALHMGALPPA

SEQ ID NO: 5 - protein, 145 aa, Artificial sequence
MGTCPLAPPGHVSGALGTLLPLAASLSAGAGGTASPICTGGVVSVSTGGATVMSCAISAAPSHVAILLAAHGGGSAIPAGVAPGTPSAAGTGLGVGGGVAGLVILGAAASHAGLTMTHLVGHGAAAAGVTLGVSGAGPGSAPATG

SEQ ID NO: 6 - protein, 4 aa, Artificial sequence
LAGL

SEQ ID NO: 7 - protein, 6 aa, Artificial sequence
SGLAGL

SEQ ID NO: 8 - protein, 240 aa, Artificial sequence
AIGMTGTTSSLSASLGAAVTISCSASGGISATLATTGGLPAGTVLLLITTTSSLHSGVPSAPSGSGSGTATSLTISALGPGAIATTTCGGTSLLPTTPGGGTLLGILAGGGGSGGGGSGGGGSGVGLVGSGGGLVLPGGSLLLSCAASGLTPSSTAMSTVAGTPGLALGTVASISSGGPTTTPASVLGAPTISAAAAAAILTLGMSSLASGATAMTTCAAAGVAGTLAVTGAGTTVTVSS

SEQ ID NO: 9 - DNA, 1116 bp, Artificial sequence
atgcagacctgccccctggcattccctggccacgtttcccaggcccttgggaccctcctgtttttggctgcctccttgagtgctcagaatgaaggctgggacagccccatctgcacagagggggtagtctctgtgtcttggggcgagaacaccgtcatgtcctgcaacatctccaacgccttctcccatgtcaacatcaagctgcgtgcccacgggcaggagagcgccatcttcaatgaggtggctccaggctacttctcccgggacggctggcagctccaggttcagggaggcgtggcacagctggtgatcaaaggcgcccgggactcccatgctgggctgtacatgtggcacctcgtgggacaccagagaaataacagacaagtcacgctggaggtttcaggtgcagaaccccagtccgcccccgacactggggcggccgcaacaactaccccagcacctcgaccaccaacaccagcacccactattgctagtcagccactgtcactgcgaccagaagcatgccgacctgcagctggaggcgctgtgcacacccggggcctggactttgcctgcgacatctatatttgggctcctctggcaggaacctgtggagtgctgctgctgagcctggtcatcacactgtattgtaagcgagggcggaagaaactgctctacattttcaaacagccttttatgagaccagtgcagacaactcaggaggaagacggctgctcctgtaggttcccagaggaagaggaagggggatgcgagctgagagtgaagttcagcaggagcgcagacgcccccgcgtaccagcagggccagaaccagctctataacgagctcaatctaggacgaagagaggagtacgatgttttggacaagagacgtggccgggaccctgagatggggggaaagccgagaaggaagaaccctcaggaaggcctgtacaatgaactgcagaaagataagatggcggaggcctacagtgagattgggatgaaaggcgagcgccggaggggcaaggggcacgatggcctttaccagggtctcagtacagccaccaaggacacctacgacgcccttcacatgcaggccctgccccctcgctaa

SEQ ID NO: 10 - DNA, 462 bp, Artificial sequence
atgcagacctgccccctggcattccctggccacgtttcccaggcccttgggaccctcctgtttttggctgcctccttgagtgctcagaatgaaggctgggacagccccatctgcacagagggggtagtctctgtgtcttggggcgagaacaccgtcatgtcctgcaacatctccaacgccttctcccatgtcaacatcaagctgcgtgcccacgggcaggagagcgccatcttcaatgaggtggctccaggctacttctcccgggacggctggcagctccaggttcagggaggcgtggcacagctggtgatcaaaggcgcccgggactcccatgctgggctgtacatgtggcacctcgtgggacaccagagaaataacagacaagtcacgctggaggtttcaggtgcagaaccccagtccgcccccgacactggggatatcagcgaaaaggacgagctgtaa

SEQ ID NO: 11 - DNA, 810 bp, Artificial sequence
atggccttaccagtgaccgccttgctcctgccgctggccttgctgctccacgccgccaggccggacatccagatgacacagactacatcctccctgtctgcctctctgggagacagagtcaccatcagttgcagtgcaagtcagggcattagcaattatttaaactggtatcagcagaaaccagatggaactgttaaactcctgatctattacacatcaagtttacactcaggagtcccatcaaggttcagtggcagtgggtctgggacagattattctctcaccatcagcaacctggaacctgaagatattgccacttattattgtcagcagtatagcaagcttccgtacacgttcggaggggggaccaagctggaaataaaacgtggaggaggaggaagcggaggaggaggatctggaggaggcgggtctgaggtgcagctggtcgaatctggaggaggactggtgaagccaggaggatctctgaaactgagttgtgccgcttcaggcctgaccttctcaagctacgccatgagctgggtgcgacagacacctgagaagcggctggaatgggtcgctagcatctcctctggcgggttcacatactatccagactccgtgaaaggcagatttactatctctcgggataacgcaagaaatattctgtacctgcagatgagttcactgaggagcgaggacaccgcaatgtactattgtgccagggacgaagtgcgcggctatctggatgtctggggagctggcactaccgtcaccgtctccagcgatatcagcgaaaaggacgagctgtaa

SEQ ID NO: 12 - protein, 21 aa, Artificial sequence
MALPVTALLLPLALLLHAAAP

SEQ ID NO: 13 - protein, 22 aa, Artificial sequence
MLLLVTSLLLCGLPHPAPLLIP

SEQ ID NO: 14 - protein, 15 aa, Artificial sequence
GGGGSGGGGSGGGGS

SEQ ID NO: 15 - protein, 18 aa, Artificial sequence
GSTSGSGLPGSGGGSTLG

SEQ ID NO: 16 - protein, 18 aa, Artificial sequence
GGAGSLLTCGAVGGAPGP

SEQ ID NO: 17 - protein, 24 aa, Artificial sequence
APVLGTLAPALLLLAGAVGSAPGP

SEQ ID NO: 18 - DNA, 1464 bp, Artificial sequence
atggctctgcccgtcaccgctctgctgctgcctctggctctgctgctgcacgccgcaagacccgacatccagatgacacagactacatcctccctgtctgcctctctgggagacagagtcaccatcagttgcagtgcaagtcagggcattagcaattatttaaactggtatcagcagaaaccagatggaactgttaaactcctgatctattacacatcaagtttacactcaggagtcccatcaaggttcagtggcagtgggtctgggacagattattctctcaccatcagcaacctggaacctgaagatattgccacttattattgtcagcagtatagcaagcttccgtacacgttcggaggggggaccaagctggaaataaaacgtggaggaggaggaagcggaggaggaggatctggaggaggcgggtctgaggtgcagctggtcgaatctggaggaggactggtgaagccaggaggatctctgaaactgagttgtgccgcttcaggcctgaccttctcaagctacgccatgagctgggtgcgacagacacctgagaagcggctggaatgggtcgctagcatctcctctggcgggttcacatactatccagactccgtgaaaggcagatttactatctctcgggataacgcaagaaatattctgtacctgcagatgagttcactgaggagcgaggacaccgcaatgtactattgtgccagggacgaagtgcgcggctatctggatgtctggggagctggcactaccgtcaccgtctccagcgcggccgcaacaactaccccagcacctcgaccaccaacaccagcacccactattgctagtcagccactgtcactgcgaccagaagcatgccgacctgcagctggaggcgctgtgcacacccggggcctggactttgcctgcgacatctatatttgggctcctctggcaggaacctgtggagtgctgctgctgagcctggtcatcacactgtattgtaagcgagggcggaagaaactgctctacattttcaaacagccttttatgagaccagtgcagacaactcaggaggaagacggctgctcctgtaggttcccagaggaagaggaagggggatgcgagctgagagtgaagttcagcaggagcgcagacgcccccgcgtaccagcagggccagaaccagctctataacgagctcaatctaggacgaagagaggagtacgatgttttggacaagagacgtggccgggaccctgagatggggggaaagccgagaaggaagaaccctcaggaaggcctgtacaatgaactgcagaaagataagatggcggaggcctacagtgagattgggatgaaaggcgagcgccggaggggcaaggggcacgatggcctttaccagggtctcagtacagccaccaaggacacctacgacgcccttcacatgcaggccctgccccctcgctaa